European Patent Application EP 4 606 383 A2, published August 27, 2025. Title: ANTI-CD3 ANTIBODY, AND MOLECULE CONTAINING SAID ANTIBODY. Applicant: DAIICHI SANKYO COMPANY, LIMITED. Application EP. The sequence listing filed with the application follows.

SEQUENCE LISTING (103 sequences)

SEQ ID NO: 1 - protein, 207 aa, Homo sapiens
MQSGTHWRVLGLCLLSVGVWGQDGNEEMGGITQTPYKVSISGTTVILTCPQYPGSEILWQHNDKNIGGDEDDKNIGSDEDHLSLKEFSELEQSGYYVCYPRGSKPEDANFYLYLRARVCENCMEMDVMSVATIVIVDICITGGLLLLVYYWSKNRKAKAKPVTRGAGAGGRQRGQNKERPPPVPNPDYEPIRKGQRDLYSGLNQRRI

SEQ ID NO: 2 - protein, 171 aa, Homo sapiens
MEHSTFLSGLVLATLLSQVSPFKIPIEELEDRVFVNCNTSITWVEGTVGTLLSDITRLDLGKRILDPRGIYRCNGTDIYKDKESTVQVHYRMCQSCVELDPATVAGIIVTDVIATLLLALGVFCFAGHETGRLSGAADTQALLRNDQVYQPLRDRDDAQYSHLGGNWARNK

SEQ ID NO: 3 - protein, 182 aa, Homo sapiens
MEQGKGLAVLILAIILLQGTLAQSIKGNHLVKVYDYQEDGSVLLTCDAEAKNITWFKDGKMIGFLTEDKKKWNLGSNAKDPRGMYQCKGSQNKSKPLQVYYRMCQNCIELNAATISGFLFAEIVSIFVLAVGVYFIAGQDGVRQSRASDKQTLLPNDQLYQPLKDREDDQYSHLQGNQLRRN

SEQ ID NO: 4 - DNA, 657 bp, synthetic construct
  misc_feature 1..657: note = CD3 epsilon gamma DNA
  source 1..657: mol_type = other DNA
atgagaggatcgcatcaccatcaccatcacggatcccagagcattaaaggtaatcacctggtgaaagtgtatgactatcaagaagatggtagcgttctgctgacctgtgatgcagaagcaaaaaacattacctggttcaaagacggcaaaatgattggttttctgaccgaagataaaaaaaaatggaatctgggcagcaatgcaaaagatccgcgtggtatgtatcagtgtaaaggtagccagaataaaagcaaaccgctgcaggtttattatcgtatgggtagcgcagatgatgcaaaaaaagatgcagccaaaaaagacgacgcgaaaaaagatgatgctaaaaaagacggttccgatggcaatgaagaaatgggtggtattacccagaccccgtataaagttagcattagcggcaccaccgttattctgacctgtccgcagtatccgggtagcgaaattctgtggcagcataacgataaaaacattggcggtgatgaggacgacaaaaatatcggtagtgatgaagatcatctgagcctgaaagaattcagcgaactggaacagagcggttattatgtttgttatcctcgtggtagcaaaccggaagatgcaaacttttatctgtatctgcgtgcacgtgttgggaagcttaat

SEQ ID NO: 5 - protein, 219 aa, synthetic construct
  REGION 1..219: note = His-scCD3 AA
MRGSHHHHHHGSQSIKGNHLVKVYDYQEDGSVLLTCDAEAKNITWFKDGKMIGFLTEDKKKWNLGSNAKDPRGMYQCKGSQNKSKPLQVYYRMGSADDAKKDAAKKDDAKKDDAKKDGSDGNEEMGGITQTPYKVSISGTTVILTCPQYPGSEILWQHNDKNIGGDEDDKNIGSDEDHLSLKEFSELEQSGYYVCYPRGSKPEDANFYLYLRARVGKLN

SEQ ID NO: 6 - DNA, 354 bp, Rutilus rutilus
  source 1..354: mol_type = genomic DNA
gaggtgcagttggtggagtctgggggaggcctggtgcagcctggaagggccctgaaactctcctgtgtagtctctggagtcacattcaattactacgggatgagctggatccgccaggctccagggaaggggctggagtgggttgcatccattactaattctggtggtagaatttactatccagactctgtgaagggccgattcactatctccagagaaaatacacaaaagaccctatacctacaaatgaacagtctgaggtctgaggacacggccacttattactgtactctcgatggtcgcgatggttgggttgcttactggggccaaggcactctggtcactgtctcttca

SEQ ID NO: 7 - protein, 118 aa, Rutilus rutilus
EVQLVESGGGLVQPGRALKLSCVVSGVTFNYYGMSWIRQAPGKGLEWVASITNSGGRIYYPDSVKGRFTISRENTQKTLYLQMNSLRSEDTATYYCTLDGRDGWVAYWGQGTLVTVSS

SEQ ID NO: 8 - DNA, 327 bp, Rutilus rutilus
  source 1..327: mol_type = genomic DNA
cagtttgtgcttactcagccaaactctgtgtctacgaatctcggaaccacagtcgaactgtcttgcaagcgcaacactgggaacattggaagcaattatgtgaactggtaccagcagcatgagggaagatctcccaccactattatttatagggatgataagagaccagatggagtttctgacaggttctctgggtccattgacagatcttccaagtcagccctcctgacaatcaataatgtgcagactgaagatgaagctgactacttctgtcagtcttacagtagtggttttattttcggcggtggaaccaagctcactgtccta

SEQ ID NO: 9 - protein, 109 aa, synthetic construct
  REGION 1..109: note = C3-147_VL AA
QFVLTQPNSVSTNLGTTVELSCKRNTGNIGSNYVNWYQQHEGRSPTTIIYRDDKRPDGVSDRFSGSIDRSSKSALLTINNVQTEDEADYFCQSYSSGFIFGGGTKLTVL

SEQ ID NO: 10 - DNA, 75 bp, synthetic construct
  misc_feature 1..75: note = G4S linker sense
  source 1..75: mol_type = other DNA
gtcactgtctcttcaggtggaggcggttcaggcggaggtggcagcggcggtggcgggagtcagtttgtgcttact

SEQ ID NO: 11 - DNA, 75 bp, synthetic construct
  misc_feature 1..75: note = G4sS linker antisense
  source 1..75: mol_type = other DNA
agtaagcacaaactgactcccgccaccgccgctgccacctccgcctgaaccgcctccacctgaagagacagtgac

SEQ ID NO: 12 - protein, 118 aa, Rutilus rutilus; identical to SEQ ID NO: 7

SEQ ID NO: 13 - protein, 109 aa, Rutilus rutilus; identical to SEQ ID NO: 9

SEQ ID NO: 14 - DNA, 867 bp, synthetic construct
  misc_feature 1..867: note = C3E-7000 ORF
  source 1..867: mol_type = other DNA
atgaaacacctgtggttcttcctcctgctggtggcagctcccagatgggtgctgagcgaggtgcagttggtggagtctgggggaggcctggtgcagcctggaagggccctgaaactctcctgtgtagtctctggagtcacattcaattactacgggatgagctggatccgccaggctccagggaaggggctggagtgggttgcatccattactaattctggtggtagaatttactatccagactctgtgaagggccgattcactatctccagagaaaatacacaaaagaccctatacctacaaatgaacagtctgaggtctgaggacacggccacttattactgtactctcgatggtcgcgatggttgggttgcttactggggccaaggcactctggtcactgtctcttcaggtggaggcggttcaggcggaggtggcagcggcggtggcgggagtcagtttgtgcttactcagccaaactctgtgtctacgaatctcggaaccacagtcgaactgtcttgcaagcgcaacactgggaacattggaagcaattatgtgaactggtaccagcagcatgagggaagatctcccaccactattatttatagggatgataagagaccagatggagtttctgacaggttctctgggtccattgacagatcttccaagtcagccctcctgacaatcaataatgtgcagactgaagatgaagctgactacttctgtcagtcttacagtagtggttttattttcggcggtggaaccaagctcactgtcctaggcgcgtctgcggccgcaggatccggtggtgattacaaagatgatgacgataaaggtgcagcggcgcatcaccatcatcaccac

SEQ ID NO: 15 - protein, 270 aa, synthetic construct
  REGION 1..270: note = C3E-7000 AA
EVQLVESGGGLVQPGRALKLSCVVSGVTFNYYGMSWIRQAPGKGLEWVASITNSGGRIYYPDSVKGRFTISRENTQKTLYLQMNSLRSEDTATYYCTLDGRDGWVAYWGQGTLVTVSSGGGGSGGGGSGGGGSQFVLTQPNSVSTNLGTTVELSCKRNTGNIGSNYVNWYQQHEGRSPTTIIYRDDKRPDGVSDRFSGSIDRSSKSALLTINNVQTEDEADYFCQSYSSGFIFGGGTKLTVLGASAAAGSGGDYKDDDDKGAAAHHHHHH

SEQ ID NO: 16 - protein, 118 aa, synthetic construct
  REGION 1..118: note = C3E-7034_VH AA
EVQLVESGGGLVQPGGSLRLSCAASGVTFNYYGMSWIRQAPGKGLEWVASITNSGGRIYYPDSVKGRFTISRENTQKTLYLQMNSLRAEDTAVYYCTLDGRDGWVAYWGQGTLVTVSS

SEQ ID NO: 17 - protein, 109 aa, synthetic construct
  REGION 1..109: note = C3E-7034_VL AA
NFMLTQPHSVSESPGKTVTISCKRNTGNIGSNYVNWYQQHEGSSPTTIIYRDDKRPDGVSDRFSGSIDRSSKSASLTISNLKTEDEADYFCQSYSSGFIFGGGTKLTVL

SEQ ID NO: 18 - DNA, 864 bp, synthetic construct
  misc_feature 1..864: note = C3E-7034 ORF
  source 1..864: mol_type = other DNA
atgaaacacctgtggttcttcctcctgctggtggcagctcccagatgggtgctgagcggagaagtgcagctggtggaatccggggggggcctggtgcagcctggggggagcctgagactgagttgtgccgcctctggggtgacatttaactactatggcatgtcttggatccgccaggcacctggaaagggcctggagtgggtggccagcatcactaattccggcgggcgaatctactatcccgacagcgtcaagggcaggttcacaatttcccgcgagaacacacagaaaactctgtacctgcagatgaatagcctgagagccgaagatacagctgtgtactattgcactctggacggcagggatgggtgggtcgcctattgggggcagggaaccctggtgacagtcagctccggaggaggaggatctggcggaggaggcagtgggggaggcgggtcaaactttatgctgacccagccccacagtgtgtcagagagccctggcaagactgtcaccatctcttgtaaaaggaacaccggaaatattggcagtaactacgtgaattggtatcagcagcatgaagggtctagtccaaccacaatcatctaccgggacgataagagacccgacggggtgtccgatcgattctccggatctatcgaccggtcaagcaagagtgcttcactgaccattagcaatctgaaaacagaggacgaagcagattacttttgccagtcctattcctctggcttcatctttggaggcgggactaaactgaccgtgctgggcgcggccgcaggtgcaggtggtgattacaaagatgatgacgataaaggtgcagcggcgcatcaccatcatcaccac

SEQ ID NO: 19 - protein, 269 aa, synthetic construct
  REGION 1..269: note = C3E-7034 AA
GEVQLVESGGGLVQPGGSLRLSCAASGVTFNYYGMSWIRQAPGKGLEWVASITNSGGRIYYPDSVKGRFTISRENTQKTLYLQMNSLRAEDTAVYYCTLDGRDGWVAYWGQGTLVTVSSGGGGSGGGGSGGGGSNFMLTQPHSVSESPGKTVTISCKRNTGNIGSNYVNWYQQHEGSSPTTIIYRDDKRPDGVSDRFSGSIDRSSKSASLTISNLKTEDEADYFCQSYSSGFIFGGGTKLTVLGAAAGAGGDYKDDDDKGAAAHHHHHH

SEQ ID NO: 20 - protein, 107 aa, synthetic construct
  REGION 1..107: note = C3E-7035_VL AA
QAVLTQPSSVSGVPGQRVTISCKRNTGNIGSNYVNWYQQLPGTAPKLLIYRDDKRPSGVPDRFSGSKSGTSASLAITGFQAEDEADYYCQSYSSGFIFGGGTKLTVL

SEQ ID NO: 21 - DNA, 864 bp, synthetic construct
  misc_feature 1..864: note = C3E-7035 ORF
  source 1..864: mol_type = other DNA
atgaaacacctgtggttcttcctcctgctggtggcagctcccagatgggtgctgagcggagaagtgcagctggtggaatccggggggggcctggtgcagcctggggggagcctgagactgagttgtgccgcctctggggtgacatttaactactatggcatgtcttggatccgccaggcacctggaaagggcctggagtgggtggccagcatcactaattccggcgggcgaatctactatcccgacagcgtcaagggcaggttcacaatttcccgcgagaacacacagaaaactctgtacctgcagatgaatagcctgagagccgaagatacagctgtgtactattgcactctggacggcagggatgggtgggtcgcctattgggggcagggaaccctggtgacagtcagctccggaggaggaggatctggcggaggaggcagtgggggaggcgggtcaatggcccaggctgtgctcactcagccgtcctctgtttctggcgtacctggccaacgggtgaccattagctgtaaaaggaataccgggaatatcgggtctaactacgtgaactggtatcagcagcttccagggacagctcccaagttgctgatctatcgcgacgacaaaagaccctcaggggtccctgaccgatttagtggcagcaaaagcggtacttccgcttccctggcgataaccggctttcaggccgaagatgaggcagactactattgccagtcatattccagcggcttcatcttcggaggcggaactaagctgacagtgctgggcgcggccgcaggtgcaggtggtgattacaaagatgatgacgataaaggtgcagcggcgcatcaccatcatcaccac

SEQ ID NO: 22 - protein, 269 aa, synthetic construct
  REGION 1..269: note = C3E-7035 AA
GEVQLVESGGGLVQPGGSLRLSCAASGVTFNYYGMSWIRQAPGKGLEWVASITNSGGRIYYPDSVKGRFTISRENTQKTLYLQMNSLRAEDTAVYYCTLDGRDGWVAYWGQGTLVTVSSGGGGSGGGGSGGGGSMAQAVLTQPSSVSGVPGQRVTISCKRNTGNIGSNYVNWYQQLPGTAPKLLIYRDDKRPSGVPDRFSGSKSGTSASLAITGFQAEDEADYYCQSYSSGFIFGGGTKLTVLGAAAGAGGDYKDDDDKGAAAHHHHHH

SEQ ID NO: 23 - protein, 107 aa, synthetic construct
  REGION 1..107: note = C3E-7036_VL AA
NFMLTQPSSVSGVPGQRVTISCTGNTGNIGSNYVNWYQQLPGTAPKLLIYRDDKRPSGVPDRFSGSKSGTSASLAITGFQAEDEADYYCQSYSSGFIFGGGTKLTVL

SEQ ID NO: 24 - DNA, 858 bp, synthetic construct
  misc_feature 1..858: note = C3E-7036 ORF
  source 1..858: mol_type = other DNA
atgaaacacctgtggttcttcctcctgctggtggcagctcccagatgggtgctgagcggagaagtgcagctggtggaatccggggggggcctggtgcagcctggggggagcctgagactgagttgtgccgcctctggggtgacatttaactactatggcatgtcttggatccgccaggcacctggaaagggcctggagtgggtggccagcatcactaattccggcgggcgaatctactatcccgacagcgtcaagggcaggttcacaatttcccgcgagaacacacagaaaactctgtacctgcagatgaatagcctgagagccgaagatacagctgtgtactattgcactctggacggcagggatgggtgggtcgcctattgggggcagggaaccctggtgacagtcagctccggaggaggaggatctggcggaggaggcagtgggggaggcgggtcaaactttatgctcactcagccgtcctctgtttctggcgtacctggccaacgggtgaccattagctgtacgggtaataccgggaatatcgggtctaactacgtgaactggtatcagcagcttccagggacagctcccaagttgctgatctatcgcgacgacaaaagaccctcaggggtccctgaccgatttagtggcagcaaaagcggtacttccgcttccctggcgataaccggctttcaggccgaagatgaggcagactactattgccagtcatattccagcggcttcatcttcggaggcggaactaagctgacagtgttgggtgcggccgcaggtgcaggtggtgattacaaagatgatgacgataaaggtgcagcggcgcatcaccatcatcaccac

SEQ ID NO: 25 - protein, 267 aa, synthetic construct
  REGION 1..267: note = C3E-7036 AA
GEVQLVESGGGLVQPGGSLRLSCAASGVTFNYYGMSWIRQAPGKGLEWVASITNSGGRIYYPDSVKGRFTISRENTQKTLYLQMNSLRAEDTAVYYCTLDGRDGWVAYWGQGTLVTVSSGGGGSGGGGSGGGGSNFMLTQPSSVSGVPGQRVTISCTGNTGNIGSNYVNWYQQLPGTAPKLLIYRDDKRPSGVPDRFSGSKSGTSASLAITGFQAEDEADYYCQSYSSGFIFGGGTKLTVLGAAAGAGGDYKDDDDKGAAAHHHHHH

SEQ ID NO: 26 - protein, 8 aa, synthetic construct
  REGION 1..8: note = 7000_CDR-H1
GVTFNYYG

SEQ ID NO: 27 - protein, 8 aa, synthetic construct
  REGION 1..8: note = 7000_CDR-H2
ITNSGGRI

SEQ ID NO: 28 - protein, 11 aa, synthetic construct
  REGION 1..11: note = 7000_CDR-H3
TLDGRDGWVAY

SEQ ID NO: 29 - protein, 8 aa, synthetic construct
  REGION 1..8: note = 7000_CDR-L1
TGNIGSNY

SEQ ID NO: 30 - skipped

SEQ ID NO: 31 - protein, 8 aa, synthetic construct
  REGION 1..8: note = 7000_CDR-L3
QSYSSGFI

SEQ ID NO: 32 - DNA, 864 bp, synthetic construct
  misc_feature 1..864: note = C3E-3000 ORF
  source 1..864: mol_type = other DNA
atgaagcacctgtggttctttctgctgctggtggccgctcccagatgggtgctgtctcaggtgcagctgcagcagtctggcgccgaactggctagacctggcgcctccgtgaagatgagctgcaaggccagcggctacaccttcacccggtacaccatgcactgggtcaagcagaggcctggacagggcctggaatggatcggctacatcaaccccagccggggctacaccaactacaaccagaagttcaaggacaaggccaccctgaccaccgacaagagcagcagcaccgcctacatgcagctgtccagcctgaccagcgaggacagcgccgtgtactactgcgcccggtactacgacgaccactactgcctggactactggggccagggcaccacactgaccgtgtctagtggtggaggcggttcaggcggaggtggcagcggcggtggcgggagtcagatcgtgctgacacagagccccgccatcatgtctgccagccctggcgagaaagtgaccatgacctgtagcgccagcagcagcgtgtcctacatgaactggtatcagcagaagtccggcaccagccccaagcggtggatctacgacacaagcaagctggcctctggcgtgcccgcccactttagaggctctggcagcggcacaagctacagcctgaccatcagcggcatggaagccgaggatgccgccacctactactgccagcagtggtccagcaaccccttcacctttggctccggcacaaagctggaaatcaagcggggcgcgtctgcggccgcaggtagcggtggtgattacaaagatgatgacgataaaggtgcagcggcgcatcaccatcatcaccac

SEQ ID NO: 33 - protein, 269 aa, synthetic construct
  REGION 1..269: note = C3E-3000 AA
QVQLQQSGAELARPGASVKMSCKASGYTFTRYTMHWVKQRPGQGLEWIGYINPSRGYTNYNQKFKDKATLTTDKSSSTAYMQLSSLTSEDSAVYYCARYYDDHYCLDYWGQGTTLTVSSGGGGSGGGGSGGGGSQIVLTQSPAIMSASPGEKVTMTCSASSSVSYMNWYQQKSGTSPKRWIYDTSKLASGVPAHFRGSGSGTSYSLTISGMEAEDAATYYCQQWSSNPFTFGSGTKLEIKRGASAAAGSGGDYKDDDDKGAAAHHHHHH

SEQ ID NO: 34 - DNA, 864 bp, synthetic construct
  misc_feature 1..864: note = C3E-3007 ORF
  source 1..864: mol_type = other DNA
atgaagcacctgtggttctttctgctgctggtggccgctcccagatgggtgctgtctcaggtgcagctggtgcagtctggcgccgagagcaaaaagcctggcgcctccgtgaaggtgtcctgcaaggccagcggctacacctttacccggtacaccatgcactgggtgcgccaggcacctggacagggcctggaatggatgggctacatcaaccccagccggggctacaccaactacaaccagaaattcaaggaccgcgtgaccatcaccgccgacaagagcaccagcaccgcctacatggaactgagcagcctgcggagcgaggacaccgccgtgtactactgtgcccggtactacgacgaccactactgcctggactactggggccagggcacactcgtgaccgtgtctagtggtggaggcggttcaggcggaggtggcagcggcggtggcgggagtcagatccagatgacccagagccctagcagcctggccgtgtctctgggagagagagccaccatcacctgtagcgccagcagcagcgtgtcctacatgaactggtatcagcagaagcccggcaaggcccccaagcggtggatctacgataccagcaagctggcctccggcgtgcccgatagattttctggcagcggctccggcaccgacttcaccctgacaatcagctccctgcaggccgaggacgtggccacctactactgtcagcagtggtccagcaaccccttcaccttcggccagggcaccaaggtggaaatcaagcggggcgcgtctgcggccgcaggtagcggtggtgattacaaagatgatgacgataaaggtgcagcggcgcatcaccatcatcaccac

SEQ ID NO: 35 - protein, 269 aa, synthetic construct
  REGION 1..269: note = C3E-3007 AA
QVQLVQSGAESKKPGASVKVSCKASGYTFTRYTMHWVRQAPGQGLEWMGYINPSRGYTNYNQKFKDRVTITADKSTSTAYMELSSLRSEDTAVYYCARYYDDHYCLDYWGQGTLVTVSSGGGGSGGGGSGGGGSQIQMTQSPSSLAVSLGERATITCSASSSVSYMNWYQQKPGKAPKRWIYDTSKLASGVPDRFSGSGSGTDFTLTISSLQAEDVATYYCQQWSSNPFTFGQGTKVEIKRGASAAAGSGGDYKDDDDKGAAAHHHHHH

SEQ ID NO: 36 - protein, 119 aa, synthetic construct [sequence omitted]

SEQ ID NO: 37 - protein, 106 aa, synthetic construct [sequence omitted]

SEQ ID NO: 38 - protein, 119 aa, synthetic construct
  REGION 1..119: note = C3E-3007_VH AA
QVQLVQSGAESKKPGASVKVSCKASGYTFTRYTMHWVRQAPGQGLEWMGYINPSRGYTNYNQKFKDRVTITADKSTSTAYMELSSLRSEDTAVYYCARYYDDHYCLDYWGQGTLVTVSS

SEQ ID NO: 39 - protein, 106 aa, synthetic construct
  REGION 1..106: note = C3E-3007_VL AA
QIQMTQSPSSLAVSLGERATITCSASSSVSYMNWYQQKPGKAPKRWIYDTSKLASGVPDRFSGSGSGTDFTLTISSLQAEDVATYYCQQWSSNPFTFGQGTKVEIK

SEQ ID NO: 40 - DNA, 822 bp, synthetic construct
  misc_feature 1..822: note = HT1-11 scFv ORF
  source 1..822: mol_type = other DNA
atgaagcacctgtggttctttctgctgctggtggccgctcccagatgggtgctgtctcaggtgcagctggtgcagtctggcgccgaagtgaagaaaccaggcgccagcgtgaaggtgtcctgcaaggccagcggctacacctttaccaccgccggcatgcagtgggtgcgccaggctcctggacagggcctggaatggatgggctggatcaacacccacagcggcgtgcccaaatacgccgaggacttcaagggcagagtgaccatcagcgccgacaccagcacctccacagcctacctgcagctgagcagcctgaagtccgaggacaccgccgtgtactactgcgccagaagcggcttcggcagcagctactggtacttcgacgtgtggggccagggcaccctcgtgacagtgtctagcggaggcggaggatctggcggcggaggaagtggcggagggggatccgatatccagatgacccagagccccagcagcctgtctgccagcgtgggcgacagagtgacaattacatgcaaggcctcccaggacgtgtccacagccgtggcctggtatcagcagaagcctggcaaggcccccaagctgctgatctacagcgccagctaccggtacaccggcgtgccaagcagattttccggcagcggctccggcaccgacttcaccctgacaatcagctccctgcagcccgaggatttcgccgtgtattattgccagcagcactacatcacccccctgaccttcggccaggggaccaagctggaaatcaagagaacaggcgccgctgcccaccaccaccatcaccat

SEQ ID NO: 41 - protein, 255 aa, synthetic construct
  REGION 1..255: note = HT1-11 scFv AA
QVQLVQSGAEVKKPGASVKVSCKASGYTFTTAGMQWVRQAPGQGLEWMGWINTHSGVPKYAEDFKGRVTISADTSTSTAYLQLSSLKSEDTAVYYCARSGFGSSYWYFDVWGQGTLVTVSSGGGGSGGGGSGGGGSDIQMTQSPSSLSASVGDRVTITCKASQDVSTAVAWYQQKPGKAPKLLIYSASYRYTGVPSRFSGSGSGTDFTLTISSLQPEDFAVYYCQQHYITPLTFGQGTKLEIKRTGAAAHHHHHH

SEQ ID NO: 42 - DNA, 1614 bp, synthetic construct
  misc_feature 1..1614: note = T2C-0001 ORF
  source 1..1614: mol_type = other DNA
atgaaacacctgtggttcttcctcctgctggtggcagctcccagatgggtgctgagcggacaggtgcagctggtgcagtctggcgccgaagtgaagaaaccaggcgccagcgtgaaggtgtcctgcaaggccagcggctacacctttaccaccgccggcatgcagtgggtgcgccaggctcctggacagggcctggaatggatgggctggatcaacacccacagcggcgtgcccaaatacgccgaggacttcaagggcagagtgaccatcagcgccgacaccagcacctccacagcctacctgcagctgagcagcctgaagtccgaggacaccgccgtgtactactgcgccagaagcggcttcggcagcagctactggtacttcgacgtgtggggccagggcaccctcgtgacagtgtctagcggaggcggaggatctggcggcggaggaagtggcggagggggatccgatatccagatgacccagagccccagcagcctgtctgccagcgtgggcgacagagtgacaattacatgcaaggcctcccaggacgtgtccacagccgtggcctggtatcagcagaagcctggcaaggcccccaagctgctgatctacagcgccagctaccggtacaccggcgtgccaagcagattttccggcagcggctccggcaccgacttcaccctgacaatcagctccctgcagcccgaggatttcgccgtgtattattgccagcagcactacatcacccccctgaccttcggccaggggaccaagctggaaatcaagagaacagggggaggcggttcagaagtgcagctggtggaatccggggggggcctggtgcagcctggggggagcctgagactgagttgtgccgcctctggggtgacatttaactactatggcatgtcttggatccgccaggcacctggaaagggcctggagtgggtggccagcatcactaattccggcgggcgaatctactatcccgacagcgtcaagggcaggttcacaatttcccgcgagaacacacagaaaactctgtacctgcagatgaatagcctgagagccgaagatacagctgtgtactattgcactctggacggcagggatgggtgggtcgcctattgggggcagggaaccctggtgacagtcagctccggaggaggaggatctggcggaggaggcagtgggggaggcgggtcaaactttatgctgacccagccccacagtgtgtcagagagccctggcaagactgtcaccatctcttgtaaaaggaacaccggaaatattggcagtaactacgtgaattggtatcagcagcatgaagggtctagtccaaccacaatcatctaccgggacgataagagacccgacggggtgtccgatcgattctccggatctatcgaccggtcaagcaagagtgcttcactgaccattagcaatctgaaaacagaggacgaagcagattacttttgccagtcctattcctctggcttcatctttggaggcgggactaaactgaccgtgctgggcgcggccgcaggtgcaggtggtgattacaaagatgatgacgataaaggtgcagcggcgcatcaccatcatcaccac

SEQ ID NO: 43 - protein, 519 aa, synthetic construct
  REGION 1..519: note = T2C-0001 AA
GQVQLVQSGAEVKKPGASVKVSCKASGYTFTTAGMQWVRQAPGQGLEWMGWINTHSGVPKYAEDFKGRVTISADTSTSTAYLQLSSLKSEDTAVYYCARSGFGSSYWYFDVWGQGTLVTVSSGGGGSGGGGSGGGGSDIQMTQSPSSLSASVGDRVTITCKASQDVSTAVAWYQQKPGKAPKLLIYSASYRYTGVPSRFSGSGSGTDFTLTISSLQPEDFAVYYCQQHYITPLTFGQGTKLEIKRTGGGGSEVQLVESGGGLVQPGGSLRLSCAASGVTFNYYGMSWIRQAPGKGLEWVASITNSGGRIYYPDSVKGRFTISRENTQKTLYLQMNSLRAEDTAVYYCTLDGRDGWVAYWGQGTLVTVSSGGGGSGGGGSGGGGSNFMLTQPHSVSESPGKTVTISCKRNTGNIGSNYVNWYQQHEGSSPTTIIYRDDKRPDGVSDRFSGSIDRSSKSASLTISNLKTEDEADYFCQSYSSGFIFGGGTKLTVLGAAAGAGGDYKDDDDKGAAAHHHHHH

SEQ ID NO: 44 - DNA, 1647 bp, synthetic construct
  misc_feature 1..1647: note = T2C-0003 ORF
  source 1..1647: mol_type = other DNA
atgaaacacctgtggttcttcctcctgctggtggcagctcccagatgggtgctgagcggacaggtgcagctggtgcagtctggcgccgaagtgaagaaaccaggcgccagcgtgaaggtgtcctgcaaggccagcggctacacctttaccaccgccggcatgcagtgggtgcgccaggctcctggacagggcctggaatggatgggctggatcaacacccacagcggcgtgcccaaatacgccgaggacttcaagggcagagtgaccatcagcgccgacaccagcacctccacagcctacctgcagctgagcagcctgaagtccgaggacaccgccgtgtactactgcgccagaagcggcttcggcagcagctactggtacttcgacgtgtggggccagggcaccctcgtgacagtgtctagcggaggcggaggatctggcggcggaggaagtggcggagggggatccgatatccagatgacccagagccccagcagcctgtctgccagcgtgggcgacagagtgacaattacatgcaaggcctcccaggacgtgtccacagccgtggcctggtatcagcagaagcctggcaaggcccccaagctgctgatctacagcgccagctaccggtacaccggcgtgccaagcagattttccggcagcggctccggcaccgacttcaccctgacaatcagctccctgcagcccgaggatttcgccgtgtattattgccagcagcactacatcacccccctgaccttcggccaggggaccaagctggaaatcaagagaacagggggaggcggttcagaagtgcagctggtggaatccggcggaggcctggtccagcctggcggcagcctgaaactgagctgcgccgccagcggcttcaccttcaacaaatacgccatgaactgggtccgccaggctcctggaaagggactcgagtgggtggcccggatcagaagcaagtacaacaactacgccacctactacgccgacagcgtgaaggaccggttcaccatcagccgggacgacagcaagaacaccgcctacctgcagatgaacaacctgaaaaccgaggacacagccgtgtactactgcgtgcggcacggcaacttcggcaacagctacatcagctactgggcctattggggacagggaacactcgtgacagtgtccagtggcggaggcggcagtggtgggggaggaagcggaggtggcggatctcagaccgtggtcacccaggaacccagcctgacagtcagccctggaggcaccgtgaccctgacctgtggaagcagcacaggcgccgtgaccagcggctactaccccaactgggtgcagcagaagcccggccaggctcctagaggcctgatcggcggcaccaagtttctggcccctggcacccctgcccggttctctggatctctgctgggcggcaaggccgccctgacactgagcggagtgcagcccgaggacgaggccgagtactactgtgccctgtggtacagcaacagatgggtgttcggcggagggaccaagctgaccgtgctgggcagcggcgcgtctgcggccgcaggtagcggtggtgattacaaagatgatgacgataaaggtgcagcggcgcatcaccatcatcaccac

SEQ ID NO: 45 - protein, 530 aa, synthetic construct
  REGION 1..530: note = T2C-0003 AA
GQVQLVQSGAEVKKPGASVKVSCKASGYTFTTAGMQWVRQAPGQGLEWMGWINTHSGVPKYAEDFKGRVTISADTSTSTAYLQLSSLKSEDTAVYYCARSGFGSSYWYFDVWGQGTLVTVSSGGGGSGGGGSGGGGSDIQMTQSPSSLSASVGDRVTITCKASQDVSTAVAWYQQKPGKAPKLLIYSASYRYTGVPSRFSGSGSGTDFTLTISSLQPEDFAVYYCQQHYITPLTFGQGTKLEIKRTGGGGSEVQLVESGGGLVQPGGSLKLSCAASGFTFNKYAMNWVRQAPGKGLEWVARIRSKYNNYATYYADSVKDRFTISRDDSKNTAYLQMNNLKTEDTAVYYCVRHGNFGNSYISYWAYWGQGTLVTVSSGGGGSGGGGSGGGGSQTVVTQEPSLTVSPGGTVTLTCGSSTGAVTSGYYPNWVQQKPGQAPRGLIGGTKFLAPGTPARFSGSLLGGKAALTLSGVQPEDEAEYYCALWYSNRWVFGGGTKLTVLGSGASAAAGSGGDYKDDDDKGAAAHHHHHH

SEQ ID NO: 46 - DNA, 1614 bp, synthetic construct
  misc_feature 1..1614: note = T2C-0005 ORF
  source 1..1614: mol_type = other DNA
atgaagcacctgtggttcttcctcctgctggtggcagctcccagatgggtgctgagcggacaggtgcagctggtgcagtctggcgccgaagtgaagaaaccaggcgccagcgtgaaggtgtcctgcaaggccagcggctacacctttaccaccgccggcatgcagtgggtgcgccaggctcctggacagggcctggaatggatgggctggatcaacacccacagcggcgtgcccaaatacgccgaggacttcaagggcagagtgaccatcagcgccgacaccagcacctccacagcctacctgcagctgagcagcctgaagtccgaggacaccgccgtgtactactgcgccagaagcggcttcggcagcagctactggtacttcgacgtgtggggccagggcaccctcgtgacagtgtctagcggaggcggaggatctggcggcggaggaagtggcggagggggatccgatatccagatgacccagagccccagcagcctgtctgccagcgtgggcgacagagtgacaattacatgcaaggcctcccaggacgtgtccacagccgtggcctggtatcagcagaagcctggcaaggcccccaagctgctgatctacagcgccagctaccggtacaccggcgtgccaagcagattttccggcagcggctccggcaccgacttcaccctgacaatcagctccctgcagcccgaggatttcgccgtgtattattgccagcagcactacatcacccccctgaccttcggccaggggaccaagctggaaatcaagagaacagggggaggcggttcagaagtgcagctggtggaatccggggggggcctggtgcagcctggggggagcctgagactgagttgtgccgcctctggggtgacatttaactactatggcatgtcttggatccgccaggcacctggaaagggcctggagtgggtggccagcatcactaattccggcgggcgaatctactatcccgacagcgtcaagggcaggttcacaatttcccgcgagaacacacagaaaactctgtacctgcagatgaatagcctgagagccgaagatacagctgtgtactattgcactctggacggcagggatgggtgggtcgcctattgggggcagggaaccctggtgacagtcagctccggaggaggaggatctggcggaggaggcagtgggggaggcgggtcaatggcccaggctgtgctcactcagccgtcctctgtttctggcgtacctggccaacgggtgaccattagctgtaaaaggaataccgggaatatcgggtctaactacgtgaactggtatcagcagcttccagggacagctcccaagttgctgatctatcgcgacgacaaaagaccctcaggggtccctgaccgatttagtggcagcaaaagcggtacttccgcttccctggcgataaccggctttcaggccgaagatgaggcagactactattgccagtcatattccagcggcttcatcttcggaggcggaactaagctgacagtgttgggcgcggccgcaggtgcaggtggtgattacaaagatgatgacgataaaggtgcagcggcgcatcaccatcatcaccac

SEQ ID NO: 47 - protein, 519 aa, synthetic construct
  REGION 1..519: note = T2C-0005 AA
GQVQLVQSGAEVKKPGASVKVSCKASGYTFTTAGMQWVRQAPGQGLEWMGWINTHSGVPKYAEDFKGRVTISADTSTSTAYLQLSSLKSEDTAVYYCARSGFGSSYWYFDVWGQGTLVTVSSGGGGSGGGGSGGGGSDIQMTQSPSSLSASVGDRVTITCKASQDVSTAVAWYQQKPGKAPKLLIYSASYRYTGVPSRFSGSGSGTDFTLTISSLQPEDFAVYYCQQHYITPLTFGQGTKLEIKRTGGGGSEVQLVESGGGLVQPGGSLRLSCAASGVTFNYYGMSWIRQAPGKGLEWVASITNSGGRIYYPDSVKGRFTISRENTQKTLYLQMNSLRAEDTAVYYCTLDGRDGWVAYWGQGTLVTVSSGGGGSGGGGSGGGGSMAQAVLTQPSSVSGVPGQRVTISCKRNTGNIGSNYVNWYQQLPGTAPKLLIYRDDKRPSGVPDRFSGSKSGTSASLAITGFQAEDEADYYCQSYSSGFIFGGGTKLTVLGAAAGAGGDYKDDDDKGAAAHHHHHH

SEQ ID NO: 48 - DNA, 1608 bp, synthetic construct
  misc_feature 1..1608: note = T2C-0006 ORF
  source 1..1608: mol_type = other DNA
atgaagcacctgtggttcttcctcctgctggtggcagctcccagatgggtgctgagcggacaggtgcagctggtgcagtctggcgccgaagtgaagaaaccaggcgccagcgtgaaggtgtcctgcaaggccagcggctacacctttaccaccgccggcatgcagtgggtgcgccaggctcctggacagggcctggaatggatgggctggatcaacacccacagcggcgtgcccaaatacgccgaggacttcaagggcagagtgaccatcagcgccgacaccagcacctccacagcctacctgcagctgagcagcctgaagtccgaggacaccgccgtgtactactgcgccagaagcggcttcggcagcagctactggtacttcgacgtgtggggccagggcaccctcgtgacagtgtctagcggaggcggaggatctggcggcggaggaagtggcggagggggatccgatatccagatgacccagagccccagcagcctgtctgccagcgtgggcgacagagtgacaattacatgcaaggcctcccaggacgtgtccacagccgtggcctggtatcagcagaagcctggcaaggcccccaagctgctgatctacagcgccagctaccggtacaccggcgtgccaagcagattttccggcagcggctccggcaccgacttcaccctgacaatcagctccctgcagcccgaggatttcgccgtgtattattgccagcagcactacatcacccccctgaccttcggccaggggaccaagctggaaatcaagagaacagggggaggcggttcagaagtgcagctggtggaatccggggggggcctggtgcagcctggggggagcctgagactgagttgtgccgcctctggggtgacatttaactactatggcatgtcttggatccgccaggcacctggaaagggcctggagtgggtggccagcatcactaattccggcgggcgaatctactatcccgacagcgtcaagggcaggttcacaatttcccgcgagaacacacagaaaactctgtacctgcagatgaatagcctgagagccgaagatacagctgtgtactattgcactctggacggcagggatgggtgggtcgcctattgggggcagggaaccctggtgacagtcagctccggaggaggaggatctggcggaggaggcagtgggggaggcgggtcaaactttatgctcactcagccgtcctctgtttctggcgtacctggccaacgggtgaccattagctgtacgggtaataccgggaatatcgggtctaactacgtgaactggtatcagcagcttccagggacagctcccaagttgctgatctatcgcgacgacaaaagaccctcaggggtccctgaccgatttagtggcagcaaaagcggtacttccgcttccctggcgataaccggctttcaggccgaagatgaggcagactactattgccagtcatattccagcggcttcatcttcggaggcggaactaagctgacagtgttgggcgcggccgcaggtgcaggtggtgattacaaagatgatgacgataaaggtgcagcggcgcatcaccatcatcaccac

SEQ ID NO: 49 - protein, 517 aa, synthetic construct
  REGION 1..517: note = T2C-0006 AA
GQVQLVQSGAEVKKPGASVKVSCKASGYTFTTAGMQWVRQAPGQGLEWMGWINTHSGVPKYAEDFKGRVTISADTSTSTAYLQLSSLKSEDTAVYYCARSGFGSSYWYFDVWGQGTLVTVSSGGGGSGGGGSGGGGSDIQMTQSPSSLSASVGDRVTITCKASQDVSTAVAWYQQKPGKAPKLLIYSASYRYTGVPSRFSGSGSGTDFTLTISSLQPEDFAVYYCQQHYITPLTFGQGTKLEIKRTGGGGSEVQLVESGGGLVQPGGSLRLSCAASGVTFNYYGMSWIRQAPGKGLEWVASITNSGGRIYYPDSVKGRFTISRENTQKTLYLQMNSLRAEDTAVYYCTLDGRDGWVAYWGQGTLVTVSSGGGGSGGGGSGGGGSNFMLTQPSSVSGVPGQRVTISCTGNTGNIGSNYVNWYQQLPGTAPKLLIYRDDKRPSGVPDRFSGSKSGTSASLAITGFQAEDEADYYCQSYSSGFIFGGGTKLTVLGAAAGAGGDYKDDDDKGAAAHHHHHH

SEQ ID NO: 50 - DNA, 37 bp, synthetic construct
  misc_feature 1..37: note = Nhe-polyC-S
  misc_feature 37: note = n is a, c, g or t
  source 1..37: mol_type = other DNA
gctagcgctaccggactcagatcccccccccccccdn

SEQ ID NO: 51 - DNA, 28 bp, synthetic construct
  misc_feature 1..28: note = rIg gamma-AS1
  source 1..28: mol_type = other DNA
tcactgagctggtgagagtgtagagccc

SEQ ID NO: 52 - DNA, 28 bp, synthetic construct
  misc_feature 1..28: note = rIg gamma-AS2
  source 1..28: mol_type = other DNA
tcaccgagctgctgagggtgtagagccc

SEQ ID NO: 53 - DNA, 37 bp, synthetic construct; identical to SEQ ID NO: 50
  misc_feature 1..37: note = Nhe-polyC-S2
  misc_feature 37: note = n is a, c, g or t
  source 1..37: mol_type = other DNA

SEQ ID NO: 54 - DNA, 26 bp, synthetic construct
  misc_feature 1..26: note = rIgL-AS1
  source 1..26: mol_type = other DNA
ttccacatcactcgggtagaaatcag

SEQ ID NO: 55 - DNA, 28 bp, synthetic construct
  misc_feature 1..28: note = rIgL-AS2
  source 1..28: mol_type = other DNA
taacaccagggtagaaatctgtcaccat

SEQ ID NO: 56 - DNA, 19 bp, synthetic construct
  misc_feature 1..19: note = rIg gamma-seq
  source 1..19: mol_type = other DNA
ctggctcagggaaatagcc

SEQ ID NO: 57 - DNA, 18 bp, synthetic construct
  misc_feature 1..18: note = rIgL-seq1
  source 1..18: mol_type = other DNA
tccctggagctcctcagt

SEQ ID NO: 58 - DNA, 18 bp, synthetic construct
  misc_feature 1..18: note = rIgL-seq2
  source 1..18: mol_type = other DNA
gccttgtcagtcttgagc

SEQ ID NO: 59 - DNA, 864 bp, synthetic construct
  misc_feature 1..864: note = C3E-7078 ORF
  source 1..864: mol_type = other DNA
atgaaacacctgtggttcttcctcctgctggtggcagctcccagatgggtgctgagcggagaagtgcagctggtggaatccggggggggcctggtgcagcctggggggagcctgagactgagttgtgccgcctctggggtgacatttaactactatggcatgtcttggatccgccaggcacctggaaagggcctggagtgggtggccagcatcactaggtccggcgggcgaatctactatcccgacagcgtcaagggcaggttcacaatttcccgcgagaacacacagaaaactctgtacctgcagatgaatagcctgagagccgaagatacagctgtgtactattgcactctggacggcagggatgggtgggtcgcctattgggggcagggaaccctggtgacagtcagctccggaggaggaggatctggcggaggaggcagtgggggaggcgggtcaaactttatgctgacccagccccacagtgtgtcagagagccctggcaagactgtcaccatctcttgtaaaaggaacaccggaaatattggcagtaactacgtgaattggtatcagcagcatgaagggtctagtccaaccacaatcatctaccgggacgataagagacccgacggggtgtccgatcgattctccggatctatcgaccggtcaagcaagagtgcttcactgaccattagcaatctgaaaacagaggacgaagcagattacttttgccagtcctattcctctggcttcatctttggaggcgggactaaactgaccgtgctgggcgcggccgcaggtgcaggtggtgattacaaagatgatgacgataaaggtgcagcggcgcatcaccatcatcaccac

SEQ ID NO: 60 - protein, 269 aa, synthetic construct
  REGION 1..269: note = C3E-7078 AA
GEVQLVESGGGLVQPGGSLRLSCAASGVTFNYYGMSWIRQAPGKGLEWVASITRSGGRIYYPDSVKGRFTISRENTQKTLYLQMNSLRAEDTAVYYCTLDGRDGWVAYWGQGTLVTVSSGGGGSGGGGSGGGGSNFMLTQPHSVSESPGKTVTISCKRNTGNIGSNYVNWYQQHEGSSPTTIIYRDDKRPDGVSDRFSGSIDRSSKSASLTISNLKTEDEADYFCQSYSSGFIFGGGTKLTVLGAAAGAGGDYKDDDDKGAAAHHHHHH

SEQ ID NO: 61 - DNA, 864 bp, synthetic construct
  misc_feature 1..864: note = C3E-7079 ORF
  source 1..864: mol_type = other DNA
atgaaacacctgtggttcttcctcctgctggtggcagctcccagatgggtgctgagcggagaagtgcagctggtggaatccggggggggcctggtgcagcctggggggagcctgagactgagttgtgccgcctctggggtgacatttaactactatggcatgtcttggatccgccaggcacctggaaagggcctggagtgggtggccagcatcacttcttccggcgggcgaatctactatcccgacagcgtcaagggcaggttcacaatttcccgcgagaacacacagaaaactctgtacctgcagatgaatagcctgagagccgaagatacagctgtgtactattgcactctggacggcagggatgggtgggtcgcctattgggggcagggaaccctggtgacagtcagctccggaggaggaggatctggcggaggaggcagtgggggaggcgggtcaaactttatgctgacccagccccacagtgtgtcagagagccctggcaagactgtcaccatctcttgtaaaaggaacaccggaaatattggcagtaactacgtgaattggtatcagcagcatgaagggtctagtccaaccacaatcatctaccgggacgataagagacccgacggggtgtccgatcgattctccggatctatcgaccggtcaagcaagagtgcttcactgaccattagcaatctgaaaacagaggacgaagcagattacttttgccagtcctattcctctggcttcatctttggaggcgggactaaactgaccgtgctgggcgcggccgcaggtgcaggtggtgattacaaagatgatgacgataaaggtgcagcggcgcatcaccatcatcaccac

SEQ ID NO: 62 - protein, 269 aa, synthetic construct
  REGION 1..269: note = C3E-7079 AA
GEVQLVESGGGLVQPGGSLRLSCAASGVTFNYYGMSWIRQAPGKGLEWVASITSSGGRIYYPDSVKGRFTISRENTQKTLYLQMNSLRAEDTAVYYCTLDGRDGWVAYWGQGTLVTVSSGGGGSGGGGSGGGGSNFMLTQPHSVSESPGKTVTISCKRNTGNIGSNYVNWYQQHEGSSPTTIIYRDDKRPDGVSDRFSGSIDRSSKSASLTISNLKTEDEADYFCQSYSSGFIFGGGTKLTVLGAAAGAGGDYKDDDDKGAAAHHHHHH

SEQ ID NO: 63 - DNA, 858 bp, synthetic construct
  misc_feature 1..858: note = C3E-7085 ORF
  source 1..858: mol_type = other DNA
atgaaacacctgtggttcttcctcctgctggtggcagctcccagatgggtgctgagcggagaagtgcagctggtggaatccggggggggcctggtgcagcctggggggagcctgagactgagttgtgccgcctctggggtgacatttaactactatggcatgtcttggatccgccaggcacctggaaagggcctggagtgggtggccagcatcactaggtccggcgggcgaatctactatcccgacagcgtcaagggcaggttcacaatttcccgcgagaacacacagaaaactctgtacctgcagatgaatagcctgagagccgaagatacagctgtgtactattgcactctggacggcagggatgggtgggtcgcctattgggggcagggaaccctggtgacagtcagctccggaggaggaggatctggcggaggaggcagtgggggaggcgggtcaaactttatgctcactcagccgtcctctgtttctggcgtacctggccaacgggtgaccattagctgtacgggtaataccgggaatatcgggtctaactacgtgaactggtatcagcagcttccagggacagctcccaagttgctgatctatcgcgacgacaaaagaccctcaggggtccctgaccgatttagtggcagcaaaagcggtacttccgcttccctggcgataaccggctttcaggccgaagatgaggcagactactattgccagtcatattccagcggcttcatcttcggaggcggaactaagctgacagtgttgggcgcggccgcaggtgcaggtggtgattacaaagatgatgacgataaaggtgcagcggcgcatcaccatcatcaccac

SEQ ID NO: 64 - protein, 267 aa, synthetic construct
  REGION 1..267: note = C3E-7085 AA
GEVQLVESGGGLVQPGGSLRLSCAASGVTFNYYGMSWIRQAPGKGLEWVASITRSGGRIYYPDSVKGRFTISRENTQKTLYLQMNSLRAEDTAVYYCTLDGRDGWVAYWGQGTLVTVSSGGGGSGGGGSGGGGSNFMLTQPSSVSGVPGQRVTISCTGNTGNIGSNYVNWYQQLPGTAPKLLIYRDDKRPSGVPDRFSGSKSGTSASLAITGFQAEDEADYYCQSYSSGFIFGGGTKLTVLGAAAGAGGDYKDDDDKGAAAHHHHHH

SEQ ID NO: 65 - DNA, 864 bp, synthetic construct
  misc_feature 1..864: note = C3E-7086 ORF
  source 1..864: mol_type = other DNA
atgaaacacctgtggttcttcctcctgctggtggcagctcccagatgggtgctgagcggagaagtgcagctggtggaatccggggggggcctggtgcagcctggggggagcctgagactgagttgtgccgcctctggggtgacatttaactactatggcatgtcttggatccgccaggcacctggaaagggcctggagtgggtggccagcatcactaggtccggcgggcgaatctactatcccgacagcgtcaagggcaggttcacaatttcccgcgagaacacacagaaaactctgtacctgcagatgaatagcctgagagccgaagatacagctgtgtactattgcactctggacggcagggatgggtgggtcgcctattgggggcagggaaccctggtgacagtcagctccggaggaggaggatctggcggaggaggcagtgggggaggcgggtcaaactttatgctgacccagccccacagtgtgtcagagagccctggcaagactgtcaccatctcttgtaaaaggaacaccggaaatattggcagtaactacgtgaattggtatcagcagcatgaagggtctagtccaaccacaatcatctaccggggcgataagagacccgacggggtgtccgatcgattctccggatctatcgaccggtcaagcaagagtgcttcactgaccattagcaatctgaaaacagaggacgaagcagattacttttgccagtcctattcctctggcttcatctttggaggcgggactaaactgaccgtgctgggcgcggccgcaggtgcaggtggtgattacaaagatgatgacgataaaggtgcagcggcgcatcaccatcatcaccac

SEQ ID NO: 66 - protein, 269 aa, synthetic construct
  REGION 1..269: note = C3E-7086 AA
GEVQLVESGGGLVQPGGSLRLSCAASGVTFNYYGMSWIRQAPGKGLEWVASITRSGGRIYYPDSVKGRFTISRENTQKTLYLQMNSLRAEDTAVYYCTLDGRDGWVAYWGQGTLVTVSSGGGGSGGGGSGGGGSNFMLTQPHSVSESPGKTVTISCKRNTGNIGSNYVNWYQQHEGSSPTTIIYRGDKRPDGVSDRFSGSIDRSSKSASLTISNLKTEDEADYFCQSYSSGFIFGGGTKLTVLGAAAGAGGDYKDDDDKGAAAHHHHHH

SEQ ID NO: 67 - DNA, 864 bp, synthetic construct
  misc_feature 1..864: note = C3E-7087 ORF
  source 1..864: mol_type = other DNA
atgaaacacctgtggttcttcctcctgctggtggcagctcccagatgggtgctgagcggagaagtgcagctggtggaatccggggggggcctggtgcagcctggggggagcctgagactgagttgtgccgcctctggggtgacatttaactactatggcatgtcttggatccgccaggcacctggaaagggcctggagtgggtggccagcatcactaggtccggcgggcgaatctactatcccgacagcgtcaagggcaggttcacaatttcccgcgagaacacacagaaaactctgtacctgcagatgaatagcctgagagccgaagatacagctgtgtactattgcactctggacggcagggatgggtgggtcgcctattgggggcagggaaccctggtgacagtcagctccggaggaggaggatctggcggaggaggcagtgggggaggcgggtcaaactttatgctgacccagccccacagtgtgtcagagagccctggcaagactgtcaccatctcttgtaaaaggaacaccggaaatattggcagtaactacgtgaattggtatcagcagcatgaagggtctagtccaaccacaatcatctaccggcaggataagagacccgacggggtgtccgatcgattctccggatctatcgaccggtcaagcaagagtgcttcactgaccattagcaatctgaaaacagaggacgaagcagattacttttgccagtcctattcctctggcttcatctttggaggcgggactaaactgaccgtgctgggcgcggccgcaggtgcaggtggtgattacaaagatgatgacgataaaggtgcagcggcgcatcaccatcatcaccac

SEQ ID NO: 68 - protein, 269 aa, synthetic construct
  REGION 1..269: note = C3E-7087 AA
GEVQLVESGGGLVQPGGSLRLSCAASGVTFNYYGMSWIRQAPGKGLEWVASITRSGGRIYYPDSVKGRFTISRENTQKTLYLQMNSLRAEDTAVYYCTLDGRDGWVAYWGQGTLVTVSSGGGGSGGGGSGGGGSNFMLTQPHSVSESPGKTVTISCKRNTGNIGSNYVNWYQQHEGSSPTTIIYRQDKRPDGVSDRFSGSIDRSSKSASLTISNLKTEDEADYFCQSYSSGFIFGGGTKLTVLGAAAGAGGDYKDDDDKGAAAHHHHHH

SEQ ID NO: 69 - DNA, 864 bp, synthetic construct
  misc_feature 1..864: note = C3E-7088 ORF
  source 1..864: mol_type = other DNA
atgaaacacctgtggttcttcctcctgctggtggcagctcccagatgggtgctgagcggagaagtgcagctggtggaatccggggggggcctggtgcagcctggggggagcctgagactgagttgtgccgcctctggggtgacatttaactactatggcatgtcttggatccgccaggcacctggaaagggcctggagtgggtggccagcatcactaggtccggcgggcgaatctactatcccgacagcgtcaagggcaggttcacaatttcccgcgagaacacacagaaaactctgtacctgcagatgaatagcctgagagccgaagatacagctgtgtactattgcactctggacggcagggatgggtgggtcgcctattgggggcagggaaccctggtgacagtcagctccggaggaggaggatctggcggaggaggcagtgggggaggcgggtcaaactttatgctgacccagccccacagtgtgtcagagagccctggcaagactgtcaccatctcttgtaaaaggaacaccggaaatattggcagtaactacgtgaattggtatcagcagcatgaagggtctagtccaaccacaatcatctaccggaacgataagagacccgacggggtgtccgatcgattctccggatctatcgaccggtcaagcaagagtgcttcactgaccattagcaatctgaaaacagaggacgaagcagattacttttgccagtcctattcctctggcttcatctttggaggcgggactaaactgaccgtgctgggcgcggccgcaggtgcaggtggtgattacaaagatgatgacgataaaggtgcagcggcgcatcaccatcatcaccac

SEQ ID NO: 70 - protein, 269 aa, synthetic construct
  REGION 1..269: note = C3E-7088 AA
GEVQLVESGGGLVQPGGSLRLSCAASGVTFNYYGMSWIRQAPGKGLEWVASITRSGGRIYYPDSVKGRFTISRENTQKTLYLQMNSLRAEDTAVYYCTLDGRDGWVAYWGQGTLVTVSSGGGGSGGGGSGGGGSNFMLTQPHSVSESPGKTVTISCKRNTGNIGSNYVNWYQQHEGSSPTTIIYRNDKRPDGVSDRFSGSIDRSSKSASLTISNLKTEDEADYFCQSYSSGFIFGGGTKLTVLGAAAGAGGDYKDDDDKGAAAHHHHHH

SEQ ID NO: 71 - DNA, 864 bp, synthetic construct
  misc_feature 1..864: note = C3E-7089 ORF
  source 1..864: mol_type = other DNA
atgaaacacctgtggttcttcctcctgctggtggcagctcccagatgggtgctgagcggagaagtgcagctggtggaatccggggggggcctggtgcagcctggggggagcctgagactgagttgtgccgcctctggggtgacatttaactactatggcatgtcttggatccgccaggcacctggaaagggcctggagtgggtggccagcatcactaggtccggcgggcgaatctactatcccgacagcgtcaagggcaggttcacaatttcccgcgagaacacacagaaaactctgtacctgcagatgaatagcctgagagccgaagatacagctgtgtactattgcactctggacggcagggatgggtgggtcgcctattgggggcagggaaccctggtgacagtcagctccggaggaggaggatctggcggaggaggcagtgggggaggcgggtcaaactttatgctgacccagccccacagtgtgtcagagagccctggcaagactgtcaccatctcttgtaaaaggaacaccggaaatattggcagtaactacgtgaattggtatcagcagcatgaagggtctagtccaaccacaatcatctaccggagcgataagagacccgacggggtgtccgatcgattctccggatctatcgaccggtcaagcaagagtgcttcactgaccattagcaatctgaaaacagaggacgaagcagattacttttgccagtcctattcctctggcttcatctttggaggcgggactaaactgaccgtgctgggcgcggccgcaggtgcaggtggtgattacaaagatgatgacgataaaggtgcagcggcgcatcaccatcatcaccac

SEQ ID NO: 72 - protein, 269 aa, synthetic construct
  REGION 1..269: note = C3E-7089 AA
GEVQLVESGGGLVQPGGSLRLSCAASGVTFNYYGMSWIRQAPGKGLEWVASITRSGGRIYYPDSVKGRFTISRENTQKTLYLQMNSLRAEDTAVYYCTLDGRDGWVAYWGQGTLVTVSSGGGGSGGGGSGGGGSNFMLTQPHSVSESPGKTVTISCKRNTGNIGSNYVNWYQQHEGSSPTTIIYRSDKRPDGVSDRFSGSIDRSSKSASLTISNLKTEDEADYFCQSYSSGFIFGGGTKLTVLGAAAGAGGDYKDDDDKGAAAHHHHHH

SEQ ID NO: 73 - DNA, 864 bp, synthetic construct
  misc_feature 1..864: note = C3E-7090 ORF
  source 1..864: mol_type = other DNA
atgaaacacctgtggttcttcctcctgctggtggcagctcccagatgggtgctgagcggagaagtgcagctggtggaatccggggggggcctggtgcagcctggggggagcctgagactgagttgtgccgcctctggggtgacatttaactactatggcatgtcttggatccgccaggcacctggaaagggcctggagtgggtggccagcatcactaggtccggcgggcgaatctactatcccgacagcgtcaagggcaggttcacaatttcccgcgagaacacacagaaaactctgtacctgcagatgaatagcctgagagccgaagatacagctgtgtactattgcactctggacggcagggatgggtgggtcgcctattgggggcagggaaccctggtgacagtcagctccggaggaggaggatctggcggaggaggcagtgggggaggcgggtcaaactttatgctgacccagccccacagtgtgtcagagagccctggcaagactgtcaccatctcttgtaaaaggaacaccggaaatattggcagtaactacgtgaattggtatcagcagcatgaagggtctagtccaaccacaatcatctaccgggccgataagagacccgacggggtgtccgatcgattctccggatctatcgaccggtcaagcaagagtgcttcactgaccattagcaatctgaaaacagaggacgaagcagattacttttgccagtcctattcctctggcttcatctttggaggcgggactaaactgaccgtgctgggcgcggccgcaggtgcaggtggtgattacaaagatgatgacgataaaggtgcagcggcgcatcaccatcatcaccac

SEQ ID NO: 74 - protein, 269 aa, synthetic construct
  REGION 1..269: note = C3E-7090 AA
GEVQLVESGGGLVQPGGSLRLSCAASGVTFNYYGMSWIRQAPGKGLEWVASITRSGGRIYYPDSVKGRFTISRENTQKTLYLQMNSLRAEDTAVYYCTLDGRDGWVAYWGQGTLVTVSSGGGGSGGGGSGGGGSNFMLTQPHSVSESPGKTVTISCKRNTGNIGSNYVNWYQQHEGSSPTTIIYRADKRPDGVSDRFSGSIDRSSKSASLTISNLKTEDEADYFCQSYSSGFIFGGGTKLTVLGAAAGAGGDYKDDDDKGAAAHHHHHH

SEQ ID NO: 75 - DNA, 864 bp, synthetic construct
  misc_feature 1..864: note = C3E-7091 ORF
  source 1..864: mol_type = other DNA
atgaaacacctgtggttcttcctcctgctggtggcagctcccagatgggtgctgagcggagaagtgcagctggtggaatccggggggggcctggtgcagcctggggggagcctgagactgagttgtgccgcctctggggtgacatttaactactatggcatgtcttggatccgccaggcacctggaaagggcctggagtgggtggccagcatcacttcttccggcgggcgaatctactatcccgacagcgtcaagggcaggttcacaatttcccgcgagaacacacagaaaactctgtacctgcagatgaatagcctgagagccgaagatacagctgtgtactattgcactctggacggcagggatgggtgggtcgcctattgggggcagggaaccctggtgacagtcagctccggaggaggaggatctggcggaggaggcagtgggggaggcgggtcaaactttatgctgacccagccccacagtgtgtcagagagccctggcaagactgtcaccatctcttgtaaaaggaacaccggaaatattggcagtaactacgtgaattggtatcagcagcatgaagggtctagtccaaccacaatcatctaccggggcgataagagacccgacggggtgtccgatcgattctccggatctatcgaccggtcaagcaagagtgcttcactgaccattagcaatctgaaaacagaggacgaagcagattacttttgccagtcctattcctctggcttcatctttggaggcgggactaaactgaccgtgctgggcgcggccgcaggtgcaggtggtgattacaaagatgatgacgataaaggtgcagcggcgcatcaccatcatcaccac

SEQ ID NO: 76 - protein, 269 aa, synthetic construct
  REGION 1..269: note = C3E-7091 AA
GEVQLVESGGGLVQPGGSLRLSCAASGVTFNYYGMSWIRQAPGKGLEWVASITSSGGRIYYPDSVKGRFTISRENTQKTLYLQMNSLRAEDTAVYYCTLDGRDGWVAYWGQGTLVTVSSGGGGSGGGGSGGGGSNFMLTQPHSVSESPGKTVTISCKRNTGNIGSNYVNWYQQHEGSSPTTIIYRGDKRPDGVSDRFSGSIDRSSKSASLTISNLKTEDEADYFCQSYSSGFIFGGGTKLTVLGAAAGAGGDYKDDDDKGAAAHHHHHH

SEQ ID NO: 77 - DNA, 864 bp, synthetic construct
  misc_feature 1..864: note = C3E-7092 ORF
  source 1..864: mol_type = other DNA
atgaaacacctgtggttcttcctcctgctggtggcagctcccagatgggtgctgagcggagaagtgcagctggtggaatccggggggggcctggtgcagcctggggggagcctgagactgagttgtgccgcctctggggtgacatttaactactatggcatgtcttggatccgccaggcacctggaaagggcctggagtgggtggccagcatcacttcttccggcgggcgaatctactatcccgacagcgtcaagggcaggttcacaatttcccgcgagaacacacagaaaactctgtacctgcagatgaatagcctgagagccgaagatacagctgtgtactattgcactctggacggcagggatgggtgggtcgcctattgggggcagggaaccctggtgacagtcagctccggaggaggaggatctggcggaggaggcagtgggggaggcgggtcaaactttatgctgacccagccccacagtgtgtcagagagccctggcaagactgtcaccatctcttgtaaaaggaacaccggaaatattggcagtaactacgtgaattggtatcagcagcatgaagggtctagtccaaccacaatcatctaccggcaggataagagacccgacggggtgtccgatcgattctccggatctatcgaccggtcaagcaagagtgcttcactgaccattagcaatctgaaaacagaggacgaagcagattacttttgccagtcctattcctctggcttcatctttggaggcgggactaaactgaccgtgctgggcgcggccgcaggtgcaggtggtgattacaaagatgatgacgataaaggtgcagcggcgcatcaccatcatcaccac

SEQ ID NO: 78 - protein, 269 aa, synthetic construct
  REGION 1..269: note = C3E-7092 AA
GEVQLVESGGGLVQPGGSLRLSCAASGVTFNYYGMSWIRQAPGKGLEWVASITSSGGRIYYPDSVKGRFTISRENTQKTLYLQMNSLRAEDTAVYYCTLDGRDGWVAYWGQGTLVTVSSGGGGSGGGGSGGGGSNFMLTQPHSVSESPGKTVTISCKRNTGNIGSNYVNWYQQHEGSSPTTIIYRQDKRPDGVSDRFSGSIDRSSKSASLTISNLKTEDEADYFCQSYSSGFIFGGGTKLTVLGAAAGAGGDYKDDDDKGAAAHHHHHH

SEQ ID NO: 79 - DNA, 864 bp, synthetic construct
  misc_feature 1..864: note = C3E-7093 ORF
  source 1..864: mol_type = other DNA
atgaaacacctgtggttcttcctcctgctggtggcagctcccagatgggtgctgagcggagaagtgcagctggtggaatccggggggggcctggtgcagcctggggggagcctgagactgagttgtgccgcctctggggtgacatttaactactatggcatgtcttggatccgccaggcacctggaaagggcctggagtgggtggccagcatcacttcttccggcgggcgaatctactatcccgacagcgtcaagggcaggttcacaatttcccgcgagaacacacagaaaactctgtacctgcagatgaatagcctgagagccgaagatacagctgtgtactattgcactctggacggcagggatgggtgggtcgcctattgggggcagggaaccctggtgacagtcagctccggaggaggaggatctggcggaggaggcagtgggggaggcgggtcaaactttatgctgacccagccccacagtgtgtcagagagccctggcaagactgtcaccatctcttgtaaaaggaacaccggaaatattggcagtaactacgtgaattggtatcagcagcatgaagggtctagtccaaccacaatcatctaccggaacgataagagacccgacggggtgtccgatcgattctccggatctatcgaccggtcaagcaagagtgcttcactgaccattagcaatctgaaaacagaggacgaagcagattacttttgccagtcctattcctctggcttcatctttggaggcgggactaaactgaccgtgctgggcgcggccgcaggtgcaggtggtgattacaaagatgatgacgataaaggtgcagcggcgcatcaccatcatcaccac

SEQ ID NO: 80 - protein, 269 aa, synthetic construct
  REGION 1..269: note = C3E-7093 AA
GEVQLVESGGGLVQPGGSLRLSCAASGVTFNYYGMSWIRQAPGKGLEWVASITSSGGRIYYPDSVKGRFTISRENTQKTLYLQMNSLRAEDTAVYYCTLDGRDGWVAYWGQGTLVTVSSGGGGSGGGGSGGGGSNFMLTQPHSVSESPGKTVTISCKRNTGNIGSNYVNWYQQHEGSSPTTIIYRNDKRPDGVSDRFSGSIDRSSKSASLTISNLKTEDEADYFCQSYSSGFIFGGGTKLTVLGAAAGAGGDYKDDDDKGAAAHHHHHH

SEQ ID NO: 81 - DNA, 864 bp, synthetic construct
  misc_feature 1..864: note = C3E-7094 ORF
  source 1..864: mol_type = other DNA
atgaaacacctgtggttcttcctcctgctggtggcagctcccagatgggtgctgagcggagaagtgcagctggtggaatccggggggggcctggtgcagcctggggggagcctgagactgagttgtgccgcctctggggtgacatttaactactatggcatgtcttggatccgccaggcacctggaaagggcctggagtgggtggccagcatcacttcttccggcgggcgaatctactatcccgacagcgtcaagggcaggttcacaatttcccgcgagaacacacagaaaactctgtacctgcagatgaatagcctgagagccgaagatacagctgtgtactattgcactctggacggcagggatgggtgggtcgcctattgggggcagggaaccctggtgacagtcagctccggaggaggaggatctggcggaggaggcagtgggggaggcgggtcaaactttatgctgacccagccccacagtgtgtcagagagccctggcaagactgtcaccatctcttgtaaaaggaacaccggaaatattggcagtaactacgtgaattggtatcagcagcatgaagggtctagtccaaccacaatcatctaccggagcgataagagacccgacggggtgtccgatcgattctccggatctatcgaccggtcaagcaagagtgcttcactgaccattagcaatctgaaaacagaggacgaagcagattacttttgccagtcctattcctctggcttcatctttggaggcgggactaaactgaccgtgctgggcgcggccgcaggtgcaggtggtgattacaaagatgatgacgataaaggtgcagcggcgcatcaccatcatcaccac

SEQ ID NO: 82 - protein, 269 aa, synthetic construct
  REGION 1..269: note = C3E-7094 AA
GEVQLVESGGGLVQPGGSLRLSCAASGVTFNYYGMSWIRQAPGKGLEWVASITSSGGRIYYPDSVKGRFTISRENTQKTLYLQMNSLRAEDTAVYYCTLDGRDGWVAYWGQGTLVTVSSGGGGSGGGGSGGGGSNFMLTQPHSVSESPGKTVTISCKRNTGNIGSNYVNWYQQHEGSSPTTIIYRSDKRPDGVSDRFSGSIDRSSKSASLTISNLKTEDEADYFCQSYSSGFIFGGGTKLTVLGAAAGAGGDYKDDDDKGAAAHHHHHH

SEQ ID NO: 83 - DNA, 864 bp, synthetic construct
  misc_feature 1..864: note = C3E-7095 ORF
  source 1..864: mol_type = other DNA
atgaaacacctgtggttcttcctcctgctggtggcagctcccagatgggtgctgagcggagaagtgcagctggtggaatccggggggggcctggtgcagcctggggggagcctgagactgagttgtgccgcctctggggtgacatttaactactatggcatgtcttggatccgccaggcacctggaaagggcctggagtgggtggccagcatcacttcttccggcgggcgaatctactatcccgacagcgtcaagggcaggttcacaatttcccgcgagaacacacagaaaactctgtacctgcagatgaatagcctgagagccgaagatacagctgtgtactattgcactctggacggcagggatgggtgggtcgcctattgggggcagggaaccctggtgacagtcagctccggaggaggaggatctggcggaggaggcagtgggggaggcgggtcaaactttatgctgacccagccccacagtgtgtcagagagccctggcaagactgtcaccatctcttgtaaaaggaacaccggaaatattggcagtaactacgtgaattggtatcagcagcatgaagggtctagtccaaccacaatcatctaccgggccgataagagacccgacggggtgtccgatcgattctccggatctatcgaccggtcaagcaagagtgcttcactgaccattagcaatctgaaaacagaggacgaagcagattacttttgccagtcctattcctctggcttcatctttggaggcgggactaaactgaccgtgctgggcgcggccgcaggtgcaggtggtgattacaaagatgatgacgataaaggtgcagcggcgcatcaccatcatcaccac

SEQ ID NO: 84 - protein, 269 aa, synthetic construct
  REGION 1..269: note = C3E-7095 AA
GEVQLVESGGGLVQPGGSLRLSCAASGVTFNYYGMSWIRQAPGKGLEWVASITSSGGRIYYPDSVKGRFTISRENTQKTLYLQMNSLRAEDTAVYYCTLDGRDGWVAYWGQGTLVTVSSGGGGSGGGGSGGGGSNFMLTQPHSVSESPGKTVTISCKRNTGNIGSNYVNWYQQHEGSSPTTIIYRADKRPDGVSDRFSGSIDRSSKSASLTISNLKTEDEADYFCQSYSSGFIFGGGTKLTVLGAAAGAGGDYKDDDDKGAAAHHHHHH

SEQ ID NO: 85 - DNA, 33 bp, synthetic construct
  misc_feature 1..33: note = HN53R Fw
  source 1..33: mol_type = other DNA
gtggccagcatcactaggtccggcgggcgaatc

SEQ ID NO: 86 - DNA, 33 bp, synthetic construct
  misc_feature 1..33: note = HN53R Rv
  source 1..33: mol_type = other DNA
gattcgcccgccggacctagtgatgctggccac

SEQ ID NO: 87 - DNA, 33 bp, synthetic construct
  misc_feature 1..33: note = HN53S Fw
  source 1..33: mol_type = other DNA
gtggccagcatcacttcttccggcgggcgaatc

SEQ ID NO: 88 - DNA, 33 bp, synthetic construct
  misc_feature 1..33: note = HN53S Rv
  source 1..33: mol_type = other DNA
gattcgcccgccggaagaagtgatgctggccac

SEQ ID NO: 89 - DNA, 1590 bp, synthetic construct
  misc_feature 1..1590: note = AXC-0001 ORF
  source 1..1590: mol_type = other DNA
atgaaacacctgtggttcttcctcctgctggtggcagctcccagatgggtgctgagcggagaagtgcagctgcaggaatctggccctggcctcgtgaagcctagccagaccctgagcctgacctgtaccgtgtccggctacagcatcaccagcaactactggggctggatcagaaagttccccggcaacaagatggaatggatcggccacatcaccaacagcggcaacaccacctacaaccccagcctgaagtcccggatcagcatcagccgggacaccagcaagaaccagttctccctgaagctgtccagcgtgacccctgccgataccgccgtgtactactgtgccaagggcgccttcgattactggggccagggaaccctcgtgaccgtgtctagcggaggcggaggatctggcggcggaggaagtggcggagggggatctgatatccagatgacccagagccccagcagcctgtctgccagcgtgggcgacagagtgaccatcacctgtagagccagccaggacatcggcaactacctgagctggttccagcagaaagtgggcaagtcccccagacggatgatctacggcgccatcaagctggccgtgggcgtgccaagcagattcagcggcagcagaagcggcagcgactacaccctgaccatcagctccctgcagcccgaggacttcgccatctactactgcctgcagtacatccagttccctctgaccttcggcagcggcaccaagctggaaatcaagagaaccgggggaggcggttcagaagtgcagctggtggaatccggggggggcctggtgcagcctggggggagcctgagactgagttgtgccgcctctggggtgacatttaactactatggcatgtcttggatccgccaggcacctggaaagggcctggagtgggtggccagcatcactaattccggcgggcgaatctactatcccgacagcgtcaagggcaggttcacaatttcccgcgagaacacacagaaaactctgtacctgcagatgaatagcctgagagccgaagatacagctgtgtactattgcactctggacggcagggatgggtgggtcgcctattgggggcagggaaccctggtgacagtcagctccggaggaggaggatctggcggaggaggcagtgggggaggcgggtcaaactttatgctgacccagccccacagtgtgtcagagagccctggcaagactgtcaccatctcttgtaaaaggaacaccggaaatattggcagtaactacgtgaattggtatcagcagcatgaagggtctagtccaaccacaatcatctaccgggacgataagagacccgacggggtgtccgatcgattctccggatctatcgaccggtcaagcaagagtgcttcactgaccattagcaatctgaaaacagaggacgaagcagattacttttgccagtcctattcctctggcttcatctttggaggcgggactaaactgaccgtgctgggcgcggccgcaggtgcaggtggtgattacaaagatgatgacgataaaggtgcagcggcgcatcaccatcatcaccac

SEQ ID NO: 90 - protein, 511 aa, synthetic construct
  REGION 1..511: note = AXC-0001 AA
GEVQLQESGPGLVKPSQTLSLTCTVSGYSITSNYWGWIRKFPGNKMEWIGHITNSGNTTYNPSLKSRISISRDTSKNQFSLKLSSVTPADTAVYYCAKGAFDYWGQGTLVTVSSGGGGSGGGGSGGGGSDIQMTQSPSSLSASVGDRVTITCRASQDIGNYLSWFQQKVGKSPRRMIYGAIKLAVGVPSRFSGSRSGSDYTLTISSLQPEDFAIYYCLQYIQFPLTFGSGTKLEIKRTGGGGSEVQLVESGGGLVQPGGSLRLSCAASGVTFNYYGMSWIRQAPGKGLEWVASITNSGGRIYYPDSVKGRFTISRENTQKTLYLQMNSLRAEDTAVYYCTLDGRDGWVAYWGQGTLVTVSSGGGGSGGGGSGGGGSNFMLTQPHSVSESPGKTVTISCKRNTGNIGSNYVNWYQQHEGSSPTTIIYRDDKRPDGVSDRFSGSIDRSSKSASLTISNLKTEDEADYFCQSYSSGFIFGGGTKLTVLGAAAGAGGDYKDDDDKGAAAHHHHHH

SEQ ID NO: 91 - DNA, 1584 bp, synthetic construct
  misc_feature 1..1584: note = AXC-0002 ORF
  source 1..1584: mol_type = other DNA
atgaaacacctgtggttcttcctcctgctggtggcagctcccagatgggtgctgagcggagaagtgcagctgcaggaatctggccctggcctcgtgaagcctagccagaccctgagcctgacctgtaccgtgtccggctacagcatcaccagcaactactggggctggatcagaaagttccccggcaacaagatggaatggatcggccacatcaccaacagcggcaacaccacctacaaccccagcctgaagtcccggatcagcatcagccgggacaccagcaagaaccagttctccctgaagctgtccagcgtgacccctgccgataccgccgtgtactactgtgccaagggcgccttcgattactggggccagggaaccctcgtgaccgtgtctagcggaggcggaggatctggcggcggaggaagtggcggagggggatctgatatccagatgacccagagccccagcagcctgtctgccagcgtgggcgacagagtgaccatcacctgtagagccagccaggacatcggcaactacctgagctggttccagcagaaagtgggcaagtcccccagacggatgatctacggcgccatcaagctggccgtgggcgtgccaagcagattcagcggcagcagaagcggcagcgactacaccctgaccatcagctccctgcagcccgaggacttcgccatctactactgcctgcagtacatccagttccctctgaccttcggcagcggcaccaagctggaaatcaagagaaccgggggaggcggttcagaagtgcagctggtggaatccggggggggcctggtgcagcctggggggagcctgagactgagttgtgccgcctctggggtgacatttaactactatggcatgtcttggatccgccaggcacctggaaagggcctggagtgggtggccagcatcactaattccggcgggcgaatctactatcccgacagcgtcaagggcaggttcacaatttcccgcgagaacacacagaaaactctgtacctgcagatgaatagcctgagagccgaagatacagctgtgtactattgcactctggacggcagggatgggtgggtcgcctattgggggcagggaaccctggtgacagtcagctccggaggaggaggatctggcggaggaggcagtgggggaggcgggtcaaactttatgctcactcagccgtcctctgtttctggcgtacctggccaacgggtgaccattagctgtacgggtaataccgggaatatcgggtctaactacgtgaactggtatcagcagcttccagggacagctcccaagttgctgatctatcgcgacgacaaaagaccctcaggggtccctgaccgatttagtggcagcaaaagcggtacttccgcttccctggcgataaccggctttcaggccgaagatgaggcagactactattgccagtcatattccagcggcttcatcttcggaggcggaactaagctgacagtgttgggcgcggccgcaggtgcaggtggtgattacaaagatgatgacgataaaggtgcagcggcgcatcaccatcatcaccac

SEQ ID NO: 92 - protein, 509 aa, synthetic construct
  REGION 1..509: note = AXC-0002 AA
GEVQLQESGPGLVKPSQTLSLTCTVSGYSITSNYWGWIRKFPGNKMEWIGHITNSGNTTYNPSLKSRISISRDTSKNQFSLKLSSVTPADTAVYYCAKGAFDYWGQGTLVTVSSGGGGSGGGGSGGGGSDIQMTQSPSSLSASVGDRVTITCRASQDIGNYLSWFQQKVGKSPRRMIYGAIKLAVGVPSRFSGSRSGSDYTLTISSLQPEDFAIYYCLQYIQFPLTFGSGTKLEIKRTGGGGSEVQLVESGGGLVQPGGSLRLSCAASGVTFNYYGMSWIRQAPGKGLEWVASITNSGGRIYYPDSVKGRFTISRENTQKTLYLQMNSLRAEDTAVYYCTLDGRDGWVAYWGQGTLVTVSSGGGGSGGGGSGGGGSNFMLTQPSSVSGVPGQRVTISCTGNTGNIGSNYVNWYQQLPGTAPKLLIYRDDKRPSGVPDRFSGSKSGTSASLAITGFQAEDEADYYCQSYSSGFIFGGGTKLTVLGAAAGAGGDYKDDDDKGAAAHHHHHH

SEQ ID NO: 93 - DNA, 1620 bp, synthetic construct
  misc_feature 1..1620: note = MGC-0001 ORF
  source 1..1620: mol_type = other DNA
atgaaacacctgtggttcttcctcctgctggtggcagctcccagatgggtgctgagcggacaggtgcagctggtgcagtctgggggaggcttggtccagcctggagggtccctgagactctcctgtgcagcctctggattcaccttcagtgactacgacatggactgggtccgccaggctccagggaaggggctggagtgggtggcagttatatcatctgatgaaaacactaaatactacgcagactccgtgaagggccgattcaccatctccagagacaattccaagaacacgctgtatctgcaaatgaacagcctgagagccgaggacacggctgtgtattactgtgcaacctataccagcacctggtatgccgttgactcctggggccagggaaccctggtcaccgtctcctcaggtggaggcggttcaggcggaggtggcagcggcggtggcgggagtgatgttgtgatgactcagtctccactctccctgcccgtcacccctggagagccggcctccatctcctgcaggtctagtcagagcctcctgcatagtaacggaaagaactatttggattggtacctgcagaagccagggcagtctccacagctcctgatctatttgggttctaatcgggcctccggggtccctgacaggttcagtggcagtggatcaggcacagattttacactgaagatcagcagagtggaggctgaggatgttggggtttattactgcatgcaaactcttcaaaccccctacacttttggccaggggaccaaggtggaaatcaaacgtgggggaggcggttcagaagtgcagctggtggaatccggggggggcctggtgcagcctggggggagcctgagactgagttgtgccgcctctggggtgacatttaactactatggcatgtcttggatccgccaggcacctggaaagggcctggagtgggtggccagcatcactaattccggcgggcgaatctactatcccgacagcgtcaagggcaggttcacaatttcccgcgagaacacacagaaaactctgtacctgcagatgaatagcctgagagccgaagatacagctgtgtactattgcactctggacggcagggatgggtgggtcgcctattgggggcagggaaccctggtgacagtcagctccggaggaggaggatctggcggaggaggcagtgggggaggcgggtcaaactttatgctgacccagccccacagtgtgtcagagagccctggcaagactgtcaccatctcttgtaaaaggaacaccggaaatattggcagtaactacgtgaattggtatcagcagcatgaagggtctagtccaaccacaatcatctaccgggacgataagagacccgacggggtgtccgatcgattctccggatctatcgaccggtcaagcaagagtgcttcactgaccattagcaatctgaaaacagaggacgaagcagattacttttgccagtcctattcctctggcttcatctttggaggcgggactaaactgaccgtgctgggcgcggccgcaggtgcaggtggtgattacaaagatgatgacgataaaggtgcagcggcgcatcaccatcatcaccac

SEQ ID NO: 94 - protein, 521 aa, synthetic construct
  REGION 1..521: note = MGC-0001 AA
GQVQLVQSGGGLVQPGGSLRLSCAASGFTFSDYDMDWVRQAPGKGLEWVAVISSDENTKYYADSVKGRFTISRDNSKNTLYLQMNSLRAEDTAVYYCATYTSTWYAVDSWGQGTLVTVSSGGGGSGGGGSGGGGSDVVMTQSPLSLPVTPGEPASISCRSSQSLLHSNGKNYLDWYLQKPGQSPQLLIYLGSNRASGVPDRFSGSGSGTDFTLKISRVEAEDVGVYYCMQTLQTPYTFGQGTKVEIKRGGGGSEVQLVESGGGLVQPGGSLRLSCAASGVTFNYYGMSWIRQAPGKGLEWVASITNSGGRIYYPDSVKGRFTISRENTQKTLYLQMNSLRAEDTAVYYCTLDGRDGWVAYWGQGTLVTVSSGGGGSGGGGSGGGGSNFMLTQPHSVSESPGKTVTISCKRNTGNIGSNYVNWYQQHEGSSPTTIIYRDDKRPDGVSDRFSGSIDRSSKSASLTISNLKTEDEADYFCQSYSSGFIFGGGTKLTVLGAAAGAGGDYKDDDDKGAAAHHHHHH

SEQ ID NO: 95 - DNA, 1614 bp, synthetic construct
  misc_feature 1..1614: note = MGC-0002 ORF
  source 1..1614: mol_type = other DNA
atgaaacacctgtggttcttcctcctgctggtggcagctcccagatgggtgctgagcggacaggtgcagctggtgcagtctgggggaggcttggtccagcctggagggtccctgagactctcctgtgcagcctctggattcaccttcagtgactacgacatggactgggtccgccaggctccagggaaggggctggagtgggtggcagttatatcatctgatgaaaacactaaatactacgcagactccgtgaagggccgattcaccatctccagagacaattccaagaacacgctgtatctgcaaatgaacagcctgagagccgaggacacggctgtgtattactgtgcaacctataccagcacctggtatgccgttgactcctggggccagggaaccctggtcaccgtctcctcaggtggaggcggttcaggcggaggtggcagcggcggtggcgggagtgatgttgtgatgactcagtctccactctccctgcccgtcacccctggagagccggcctccatctcctgcaggtctagtcagagcctcctgcatagtaacggaaagaactatttggattggtacctgcagaagccagggcagtctccacagctcctgatctatttgggttctaatcgggcctccggggtccctgacaggttcagtggcagtggatcaggcacagattttacactgaagatcagcagagtggaggctgaggatgttggggtttattactgcatgcaaactcttcaaaccccctacacttttggccaggggaccaaggtggaaatcaaacgtgggggaggcggttcagaagtgcagctggtggaatccggggggggcctggtgcagcctggggggagcctgagactgagttgtgccgcctctggggtgacatttaactactatggcatgtcttggatccgccaggcacctggaaagggcctggagtgggtggccagcatcactaattccggcgggcgaatctactatcccgacagcgtcaagggcaggttcacaatttcccgcgagaacacacagaaaactctgtacctgcagatgaatagcctgagagccgaagatacagctgtgtactattgcactctggacggcagggatgggtgggtcgcctattgggggcagggaaccctggtgacagtcagctccggaggaggaggatctggcggaggaggcagtgggggaggcgggtcaaactttatgctcactcagccgtcctctgtttctggcgtacctggccaacgggtgaccattagctgtacgggtaataccgggaatatcgggtctaactacgtgaactggtatcagcagcttccagggacagctcccaagttgctgatctatcgcgacgacaaaagaccctcaggggtccctgaccgatttagtggcagcaaaagcggtacttccgcttccctggcgataaccggctttcaggccgaagatgaggcagactactattgccagtcatattccagcggcttcatcttcggaggcggaactaagctgacagtgttgggcgcggccgcaggtgcaggtggtgattacaaagatgatgacgataaaggtgcagcggcgcatcaccatcatcaccac

SEQ ID NO: 96 - protein, 519 aa, synthetic construct
  REGION 1..519: note = MGC-0002 AA
GQVQLVQSGGGLVQPGGSLRLSCAASGFTFSDYDMDWVRQAPGKGLEWVAVISSDENTKYYADSVKGRFTISRDNSKNTLYLQMNSLRAEDTAVYYCATYTSTWYAVDSWGQGTLVTVSSGGGGSGGGGSGGGGSDVVMTQSPLSLPVTPGEPASISCRSSQSLLHSNGKNYLDWYLQKPGQSPQLLIYLGSNRASGVPDRFSGSGSGTDFTLKISRVEAEDVGVYYCMQTLQTPYTFGQGTKVEIKRGGGGSEVQLVESGGGLVQPGGSLRLSCAASGVTFNYYGMSWIRQAPGKGLEWVASITNSGGRIYYPDSVKGRFTISRENTQKTLYLQMNSLRAEDTAVYYCTLDGRDGWVAYWGQGTLVTVSSGGGGSGGGGSGGGGSNFMLTQPSSVSGVPGQRVTISCTGNTGNIGSNYVNWYQQLPGTAPKLLIYRDDKRPSGVPDRFSGSKSGTSASLAITGFQAEDEADYYCQSYSSGFIFGGGTKLTVLGAAAGAGGDYKDDDDKGAAAHHHHHH

SEQ ID NO: 97 - protein, 10 aa, Homo sapiens
ILFGISLREV

SEQ ID NO: 98 - protein, 8 aa, synthetic construct
  REGION 1..8: note = CDRH2 of variants
  SITE 3: note = Xaa - the first Xaa is any naturally occurring amino acid
  SITE 4: note = Xaa - the second Xaa is any naturally occurring amino acid
ITXXGGRI

SEQ ID NO: 99 - skipped

SEQ ID NO: 100 - protein, 118 aa, synthetic construct
  REGION 1..118: note = VH of C3E-7034 variants
  SITE 53: note = MISC_FEATURE - The first Xaa is any naturally occurring amino acid
  SITE 54: note = MISC_FEATURE - The second Xaa is any naturally occurring amino acid
EVQLVESGGGLVQPGGSLRLSCAASGVTFNYYGMSWIRQAPGKGLEWVASITXXGGRIYYPDSVKGRFTISRENTQKTLYLQMNSLRAEDTAVYYCTLDGRDGWVAYWGQGTLVTVSS

SEQ ID NO: 101 - protein, 109 aa, synthetic construct
  REGION 1..109: note = VL of C3E-7034 variants
  SITE 52: note = MISC_FEATURE - Xaa is any naturally occurring amino acid
NFMLTQPHSVSESPGKTVTISCKRNTGNIGSNYVNWYQQHEGSSPTTIIYRXDKRPDGVSDRFSGSIDRSSKSASLTISNLKTEDEADYFCQSYSSGFIFGGGTKLTVL

SEQ ID NO: 102 - protein, 107 aa, synthetic construct
  REGION 1..107: note = VL of C3E-7035 variants
  SITE 52: note = MISC_FEATURE - Xaa is any naturally occurring amino acid
QAVLTQPSSVSGVPGQRVTISCKRNTGNIGSNYVNWYQQLPGTAPKLLIYRXDKRPSGVPDRFSGSKSGTSASLAITGFQAEDEADYYCQSYSSGFIFGGGTKLTVL

SEQ ID NO: 103 - protein, 107 aa, synthetic construct
  REGION 1..107: note = VL of C3E-7036 variants
  SITE 52: note = MISC_FEATURE - Xaa is any naturally occurring amino acid
NFMLTQPSSVSGVPGQRVTISCTGNTGNIGSNYVNWYQQLPGTAPKLLIYRXDKRPSGVPDRFSGSKSGTSASLAITGFQAEDEADYYCQSYSSGFIFGGGTKLTVL